European Patent Specification EP 4 048 829 B1, published June 10, 2026. Title: SAMPLE PREPARATION AND SEQUENCING ANALYSIS FOR REPEAT EXPANSION DISORDERS AND SHORT READ DEFICIENT TARGETS. Applicant: JUMPCODE GENOMICS, INC. Application EP 20879694.6. The sequence listing filed with the application follows.

SEQUENCE LISTING (4 sequences)

SEQ ID NO: 1 - DNA, 21 bp, Homo sapiens
cattcacaggtaatcatgcta

SEQ ID NO: 2 - protein, 7 aa, Homo sapiens
HSQVIML

SEQ ID NO: 3 - DNA, 21 bp, Homo sapiens
cattcacagcagcaggtaatc

SEQ ID NO: 4 - protein, 7 aa, Homo sapiens
HSQQQVI